European Patent Application EP 4 119 166 A1, published January 18, 2023. Title: Composition For Inducing Death of Cells Having Genomic Sequence Variations And Method For Inducing Death of Cells Having Genomic Sequence Variations Using the Same. Applicant: Institute for Basic Science Ulsan National Institute of Science and Technology. The sequence listing filed with the application follows.

SEQUENCE LISTING (254 sequences)

SEQ ID NO: 1 - DNA, 21 bp, Artificial Sequence
  Polynucleotide coding gRNA
tacctatgcctcatgtagaaa

SEQ ID NO: 2 - DNA, 21 bp, Artificial Sequence
  Polynucleotide coding gRNA
atcgtcaggttctgggaccgt

SEQ ID NO: 3 - DNA, 21 bp, Artificial Sequence
  Polynucleotide coding gRNA
cagaagagagagagtagtaga

SEQ ID NO: 4 - DNA, 21 bp, Artificial Sequence
  Polynucleotide coding gRNA
gaatgtttaaggtatagttta

SEQ ID NO: 5 - DNA, 21 bp, Artificial Sequence
  Polynucleotide coding gRNA
tgtttcagcaggggttgaagc

SEQ ID NO: 6 - DNA, 21 bp, Artificial Sequence
  Polynucleotide coding gRNA
ctataccctagacttattcct

SEQ ID NO: 7 - DNA, 21 bp, Artificial Sequence
  Polynucleotide coding gRNA
gtttctttctacagaatagag

SEQ ID NO: 8 - DNA, 21 bp, Artificial Sequence
  Polynucleotide coding gRNA
ataggttaacaaagatattca

SEQ ID NO: 9 - DNA, 21 bp, Artificial Sequence
  Polynucleotide coding gRNA
ctacaaaataggtgacataac

SEQ ID NO: 10 - DNA, 21 bp, Artificial Sequence
  Polynucleotide coding gRNA
ttaaaatggcgcaaataaatt

SEQ ID NO: 11 - DNA, 21 bp, Artificial Sequence
  Polynucleotide coding gRNA
ttttatgagtctgccaggaat

SEQ ID NO: 12 - DNA, 21 bp, Artificial Sequence
  Polynucleotide coding gRNA
gaagaaacaattttcactggg

SEQ ID NO: 13 - DNA, 21 bp, Artificial Sequence
  Polynucleotide coding gRNA
caggaagggagctagtgagct

SEQ ID NO: 14 - DNA, 21 bp, Artificial Sequence
  Polynucleotide coding gRNA
cctctcctgctgatgatcccc

SEQ ID NO: 15 - DNA, 21 bp, Artificial Sequence
  Polynucleotide coding gRNA
tgggccgcacgtgtgagtgcc

SEQ ID NO: 16 - DNA, 21 bp, Artificial Sequence
  Polynucleotide coding gRNA
aggaaacaagcccatgttccc

SEQ ID NO: 17 - DNA, 21 bp, Artificial Sequence
  Polynucleotide coding gRNA
catggcagaaaacagaagaca

SEQ ID NO: 18 - DNA, 21 bp, Artificial Sequence
  Polynucleotide coding gRNA
aacagtctctgtgatagggca

SEQ ID NO: 19 - DNA, 21 bp, Artificial Sequence
  Polynucleotide coding gRNA
gggaaaatcagacggatattc

SEQ ID NO: 20 - DNA, 21 bp, Artificial Sequence
  Polynucleotide coding gRNA
atttctgttcttccctcactt

SEQ ID NO: 21 - DNA, 21 bp, Artificial Sequence
  Polynucleotide coding gRNA
taataactgtgtagttataac

SEQ ID NO: 22 - DNA, 21 bp, Artificial Sequence
  Polynucleotide coding gRNA
gttcagattagctcttaacta

SEQ ID NO: 23 - DNA, 21 bp, Artificial Sequence
  Polynucleotide coding gRNA
taaacttcctatttattgtct

SEQ ID NO: 24 - DNA, 21 bp, Artificial Sequence
  Polynucleotide coding gRNA
ataactaatgccagggtgagt

SEQ ID NO: 25 - DNA, 21 bp, Artificial Sequence
  Polynucleotide coding gRNA
ctccacgccggtagggttaga

SEQ ID NO: 26 - DNA, 21 bp, Artificial Sequence
  Polynucleotide coding gRNA
agtttgtagtgtctttccaga

SEQ ID NO: 27 - DNA, 21 bp, Artificial Sequence
  Polynucleotide coding gRNA
tattttccagatgttccaata

SEQ ID NO: 28 - DNA, 21 bp, Artificial Sequence
  Polynucleotide coding gRNA
gactatgagactactactgca

SEQ ID NO: 29 - DNA, 21 bp, Artificial Sequence
  Polynucleotide coding gRNA
ccttagcctccttttcacaca

SEQ ID NO: 30 - DNA, 21 bp, Artificial Sequence
  Polynucleotide coding gRNA
agagaagagaaaataggggaa

SEQ ID NO: 31 - protein, 475 aa, Artificial Sequence
  Exonuclease I
MMNDGKQQSTFLFHDYETFGTHPALDRPAQFAAIRTDSEFNVIGEPEVFYCKPADDYLPQPGAVLITGITPQEARAKGENEAAFAARIHSLFTVPKTCILGYNNVRFDDEVTRNIFYRNFYDPYAWSWQHDNSRWDLLDVMRACYALRPEGINWPENDDGLPSFRLEHLTKANGIEHSNAHDAMADVYATIAMAKLVKTRQPRLFDYLFTHRNKHKLMALIDVPQMKPLVHVSGMFGAWRGNTSWVAPLAWHPENRNAVIMVDLAGDISPLLELDSDTLRERLYTAKTDLGDNAAVPVKLVHINKCPVLAQANTLRPEDADRLGINRQHCLDNLKILRENPQVREKVVAIFAEAEPFTPSDNVDAQLYNGFFSDADRAAMKIVLETEPRNLPALDITFVDKRIEKLLFNYRARNFPGTLDYAEQQRWLEHRRQVFTPEFLQGYADELQMLVQQYADDKEKVALLKALWQYAEEIV

SEQ ID NO: 32 - DNA, 20 bp, Artificial Sequence
  Polynucleotide coding gRNA
gaagccgacgtacactgaaa

SEQ ID NO: 33 - DNA, 20 bp, Artificial Sequence
  Polynucleotide coding gRNA
gctccgatcgggttacaaca

SEQ ID NO: 34 - DNA, 20 bp, Artificial Sequence
  Polynucleotide coding gRNA
tgacatcaattattatacat

SEQ ID NO: 35 - DNA, 20 bp, Artificial Sequence
  Polynucleotide coding gRNA
aggtgtggttccagaaccgg

SEQ ID NO: 36 - DNA, 20 bp, Artificial Sequence
  Polynucleotide coding gRNA
aactacacggagagcaagag

SEQ ID NO: 37 - DNA, 20 bp, Artificial Sequence
  Polynucleotide coding gRNA
acgccattgttaatgcacgg

SEQ ID NO: 38 - DNA, 20 bp, Artificial Sequence
  Polynucleotide coding gRNA
gcaactggagcctcagatga

SEQ ID NO: 39 - DNA, 20 bp, Artificial Sequence
  Polynucleotide coding gRNA
actcaggaggctgatgtgga

SEQ ID NO: 40 - DNA, 20 bp, Artificial Sequence
  Polynucleotide coding gRNA
gaacatgtccgaacatcaga

SEQ ID NO: 41 - DNA, 20 bp, Artificial Sequence
  Polynucleotide coding gRNA
ggagactcatctaacacata

SEQ ID NO: 42 - DNA, 20 bp, Artificial Sequence
  Polynucleotide coding gRNA
cctagctactcggtaggctg

SEQ ID NO: 43 - DNA, 20 bp, Artificial Sequence
  Polynucleotide coding gRNA
taagtaggaatgcctagagt

SEQ ID NO: 44 - DNA, 20 bp, Artificial Sequence
  Polynucleotide coding gRNA
gcaggcaagagaacatgtgc

SEQ ID NO: 45 - DNA, 20 bp, Artificial Sequence
  Polynucleotide coding gRNA
gaacacttacacactgctgg

SEQ ID NO: 46 - DNA, 20 bp, Artificial Sequence
  Polynucleotide coding gRNA
gaggttacagtgagctatga

SEQ ID NO: 47 - DNA, 20 bp, Artificial Sequence
  Polynucleotide coding gRNA
tgtcttgtgcagttgagata

SEQ ID NO: 48 - DNA, 20 bp, Artificial Sequence
  Polynucleotide coding gRNA
gcagaggcaggtggatcatg

SEQ ID NO: 49 - DNA, 20 bp, Artificial Sequence
  Polynucleotide coding gRNA
gcaacctctagagtcggcat

SEQ ID NO: 50 - DNA, 20 bp, Artificial Sequence
  Polynucleotide coding gRNA
gagaattgcttgaatgcagg

SEQ ID NO: 51 - DNA, 20 bp, Artificial Sequence
  Polynucleotide coding gRNA
aggttgcctgttgactctga

SEQ ID NO: 52 - DNA, 20 bp, Artificial Sequence
  Polynucleotide coding gRNA
ggaagaacattccatgctcg

SEQ ID NO: 53 - DNA, 20 bp, Artificial Sequence
  Polynucleotide coding gRNA
gaatagtgagttgtggagga

SEQ ID NO: 54 - DNA, 20 bp, Artificial Sequence
  Polynucleotide coding gRNA
tgagaccagcatggccaaca

SEQ ID NO: 55 - DNA, 20 bp, Artificial Sequence
  Polynucleotide coding gRNA
tactcaagcctcagtaatgg

SEQ ID NO: 56 - DNA, 20 bp, Artificial Sequence
  Polynucleotide coding gRNA
agagtgcagtggcgcgatct

SEQ ID NO: 57 - DNA, 20 bp, Artificial Sequence
  Polynucleotide coding gRNA
gaagtcaagaattgaggttt

SEQ ID NO: 58 - DNA, 20 bp, Artificial Sequence
  Polynucleotide coding gRNA
caggagaatcacttgaacct

SEQ ID NO: 59 - DNA, 21 bp, Artificial Sequence
  Polynucleotide coding gRNA
gttcatggccagaaggacgaa

SEQ ID NO: 60 - DNA, 21 bp, Artificial Sequence
  Polynucleotide coding gRNA
ataatagtgcaatcaataaaa

SEQ ID NO: 61 - DNA, 21 bp, Artificial Sequence
  Polynucleotide coding gRNA
ggaccgtcaaataaagaagta

SEQ ID NO: 62 - DNA, 21 bp, Artificial Sequence
  Polynucleotide coding gRNA
ttcccaggtgttagggtgtta

SEQ ID NO: 63 - DNA, 21 bp, Artificial Sequence
  Polynucleotide coding gRNA
aacaaaaatatcaaaccccca

SEQ ID NO: 64 - DNA, 21 bp, Artificial Sequence
  Polynucleotide coding gRNA
cttcctcccggtgacggtgac

SEQ ID NO: 65 - DNA, 21 bp, Artificial Sequence
  Polynucleotide coding gRNA
gtcggaggcaaggagagctca

SEQ ID NO: 66 - DNA, 21 bp, Artificial Sequence
  Polynucleotide coding gRNA
cagccacagaagactctgtct

SEQ ID NO: 67 - DNA, 21 bp, Artificial Sequence
  Polynucleotide coding gRNA
tcagcagctttgagaagctgt

SEQ ID NO: 68 - DNA, 21 bp, Artificial Sequence
  Polynucleotide coding gRNA
tttggctttaattcagccata

SEQ ID NO: 69 - DNA, 21 bp, Artificial Sequence
  Polynucleotide coding gRNA
aaaaaatgtgctgcattagta

SEQ ID NO: 70 - DNA, 21 bp, Artificial Sequence
  Polynucleotide coding gRNA
agacagccttcggcattgctt

SEQ ID NO: 71 - DNA, 21 bp, Artificial Sequence
  Polynucleotide coding gRNA
ggacccacaagaaaaggcatc

SEQ ID NO: 72 - DNA, 21 bp, Artificial Sequence
  Polynucleotide coding gRNA
atattccacaggtatatgcaa

SEQ ID NO: 73 - DNA, 21 bp, Artificial Sequence
  Polynucleotide coding gRNA
gatggtatcatgaggtcttaa

SEQ ID NO: 74 - DNA, 21 bp, Artificial Sequence
  Polynucleotide coding gRNA
agttgtacaatagacgagcat

SEQ ID NO: 75 - DNA, 21 bp, Artificial Sequence
  Polynucleotide coding gRNA
tgttgtgtgggcatcaccttg

SEQ ID NO: 76 - DNA, 21 bp, Artificial Sequence
  Polynucleotide coding gRNA
tgatttagttcttcatgctgt

SEQ ID NO: 77 - DNA, 21 bp, Artificial Sequence
  Polynucleotide coding gRNA
catttgacaatcagattataa

SEQ ID NO: 78 - DNA, 21 bp, Artificial Sequence
  Polynucleotide coding gRNA
gtctggggaatataagttttt

SEQ ID NO: 79 - DNA, 21 bp, Artificial Sequence
  Polynucleotide coding gRNA
aacaaatctttaagcacttga

SEQ ID NO: 80 - DNA, 21 bp, Artificial Sequence
  Polynucleotide coding gRNA
ccagagtagggcatcatccca

SEQ ID NO: 81 - DNA, 21 bp, Artificial Sequence
  Polynucleotide coding gRNA
tataaaaatatgcaaactaaa

SEQ ID NO: 82 - DNA, 21 bp, Artificial Sequence
  Polynucleotide coding gRNA
cgacgagagcttagccagagt

SEQ ID NO: 83 - DNA, 21 bp, Artificial Sequence
  Polynucleotide coding gRNA
ggcttaaacgtttctaggaca

SEQ ID NO: 84 - DNA, 21 bp, Artificial Sequence
  Polynucleotide coding gRNA
tatgtagctattgactgacaa

SEQ ID NO: 85 - DNA, 21 bp, Artificial Sequence
  Polynucleotide coding gRNA
aatttagctgtagaattatgt

SEQ ID NO: 86 - DNA, 21 bp, Artificial Sequence
  Polynucleotide coding gRNA
ctgaaatttcagcttatgaat

SEQ ID NO: 87 - DNA, 21 bp, Artificial Sequence
  Polynucleotide coding gRNA
atctgaaatattgacactctt

SEQ ID NO: 88 - DNA, 21 bp, Artificial Sequence
  Polynucleotide coding gRNA
caaatgaccttgtgattgata

SEQ ID NO: 89 - DNA, 21 bp, Artificial Sequence
  Polynucleotide coding gRNA
tttggaagtgctctcatcagt

SEQ ID NO: 90 - DNA, 21 bp, Artificial Sequence
  Polynucleotide coding gRNA
tgaaagatgcttaagttactt

SEQ ID NO: 91 - DNA, 21 bp, Artificial Sequence
  Polynucleotide coding gRNA
cacctaggaatcctcagttca

SEQ ID NO: 92 - DNA, 21 bp, Artificial Sequence
  Polynucleotide coding gRNA
tggttttcgttagtttaatta

SEQ ID NO: 93 - DNA, 21 bp, Artificial Sequence
  Polynucleotide coding gRNA
tcataagattcaaaaagaata

SEQ ID NO: 94 - DNA, 21 bp, Artificial Sequence
  Polynucleotide coding gRNA
tggcaatgtggtgaatgaagt

SEQ ID NO: 95 - DNA, 21 bp, Artificial Sequence
  Polynucleotide coding gRNA
aaggcattatgtaaacagatc

SEQ ID NO: 96 - DNA, 21 bp, Artificial Sequence
  Polynucleotide coding gRNA
agtcattaatttcttctgaga

SEQ ID NO: 97 - DNA, 21 bp, Artificial Sequence
  Polynucleotide coding gRNA
tttaaaattatcagtctaagt

SEQ ID NO: 98 - DNA, 21 bp, Artificial Sequence
  Polynucleotide coding gRNA
tcaccatttaaatataaggaa

SEQ ID NO: 99 - DNA, 21 bp, Artificial Sequence
  Polynucleotide coding gRNA
tagcaataaagactattacat

SEQ ID NO: 100 - DNA, 21 bp, Artificial Sequence
  Polynucleotide coding gRNA
tggaaataaagcttgttaagt

SEQ ID NO: 101 - DNA, 21 bp, Artificial Sequence
  Polynucleotide coding gRNA
ttctagttaacaggattgata

SEQ ID NO: 102 - DNA, 21 bp, Artificial Sequence
  Polynucleotide coding gRNA
aaaaacgtaaaaaatggaaat

SEQ ID NO: 103 - DNA, 21 bp, Artificial Sequence
  Polynucleotide coding gRNA
ctgaaccctttttctacatga

SEQ ID NO: 104 - DNA, 21 bp, Artificial Sequence
  Polynucleotide coding gRNA
gtaataaagggaaaataacct

SEQ ID NO: 105 - DNA, 21 bp, Artificial Sequence
  Polynucleotide coding gRNA
ttcctcctgttttagcaagta

SEQ ID NO: 106 - DNA, 21 bp, Artificial Sequence
  Polynucleotide coding gRNA
tcagattagctcttaactata

SEQ ID NO: 107 - DNA, 21 bp, Artificial Sequence
  Polynucleotide coding gRNA
ggtttaaagcagaacagacta

SEQ ID NO: 108 - DNA, 21 bp, Artificial Sequence
  Polynucleotide coding gRNA
ctgctgaatgaactacgctgt

SEQ ID NO: 109 - DNA, 21 bp, Artificial Sequence
  Polynucleotide coding gRNA
actaatctcttcttctatagt

SEQ ID NO: 110 - DNA, 21 bp, Artificial Sequence
  Polynucleotide coding gRNA
cttggtttgctcaaagtaatt

SEQ ID NO: 111 - DNA, 21 bp, Artificial Sequence
  Polynucleotide coding gRNA
cagtctgtaatagttagtttt

SEQ ID NO: 112 - DNA, 21 bp, Artificial Sequence
  Polynucleotide coding gRNA
tcttgtcctgaggtaacttgt

SEQ ID NO: 113 - DNA, 21 bp, Artificial Sequence
  Polynucleotide coding gRNA
agccagagatcctgcaacggt

SEQ ID NO: 114 - DNA, 21 bp, Artificial Sequence
  Polynucleotide coding gRNA
catgcagagaatgtggccaga

SEQ ID NO: 115 - DNA, 21 bp, Artificial Sequence
  Polynucleotide coding gRNA
aacagattttttaataaactc

SEQ ID NO: 116 - DNA, 21 bp, Artificial Sequence
  Polynucleotide coding gRNA
tttgagaagctgtgggcgaga

SEQ ID NO: 117 - DNA, 21 bp, Artificial Sequence
  Polynucleotide coding gRNA
taatctcaacccaaaaaataa

SEQ ID NO: 118 - DNA, 21 bp, Artificial Sequence
  Polynucleotide coding gRNA
caccagtggtcttttcctcag

SEQ ID NO: 119 - DNA, 21 bp, Artificial Sequence
  Polynucleotide coding gRNA
ctagaaacaactctcaagaca

SEQ ID NO: 120 - DNA, 21 bp, Artificial Sequence
  Polynucleotide coding gRNA
gaagggaaaaattcagcctct

SEQ ID NO: 121 - DNA, 21 bp, Artificial Sequence
  Polynucleotide coding gRNA
ctgctgggtcctgtggttaga

SEQ ID NO: 122 - DNA, 21 bp, Artificial Sequence
  Polynucleotide coding gRNA
ggctaaaggattgatttgatt

SEQ ID NO: 123 - DNA, 21 bp, Artificial Sequence
  Polynucleotide coding gRNA
gattctaactagatagttatt

SEQ ID NO: 124 - DNA, 21 bp, Artificial Sequence
  Polynucleotide coding gRNA
cctgaaacacttcttctagat

SEQ ID NO: 125 - DNA, 21 bp, Artificial Sequence
  Polynucleotide coding gRNA
ggtgcactttacaagcagcac

SEQ ID NO: 126 - DNA, 21 bp, Artificial Sequence
  Polynucleotide coding gRNA
atttattgggcgattgataaa

SEQ ID NO: 127 - DNA, 21 bp, Artificial Sequence
  Polynucleotide coding gRNA
tggagctggccctcttgtaac

SEQ ID NO: 128 - DNA, 21 bp, Artificial Sequence
  Polynucleotide coding gRNA
gaagttatctttaaaactaag

SEQ ID NO: 129 - DNA, 21 bp, Artificial Sequence
  Polynucleotide coding gRNA
ggtgagataagaataagcctt

SEQ ID NO: 130 - DNA, 21 bp, Artificial Sequence
  Polynucleotide coding gRNA
ttgtattaagaagaggttctc

SEQ ID NO: 131 - DNA, 21 bp, Artificial Sequence
  Polynucleotide coding gRNA
gaggttttctcttaagcatgt

SEQ ID NO: 132 - DNA, 21 bp, Artificial Sequence
  Polynucleotide coding gRNA
actttatcaaatgtaaaatca

SEQ ID NO: 133 - DNA, 21 bp, Artificial Sequence
  Polynucleotide coding gRNA
agtgagcaatgcatcaggtta

SEQ ID NO: 134 - DNA, 21 bp, Artificial Sequence
  Polynucleotide coding gRNA
ctagcctttcttacagtttat

SEQ ID NO: 135 - DNA, 21 bp, Artificial Sequence
  Polynucleotide coding gRNA
cctaaaaaatcaaatacccag

SEQ ID NO: 136 - DNA, 21 bp, Artificial Sequence
  Polynucleotide coding gRNA
ggaaaataaataaaaatgtgt

SEQ ID NO: 137 - DNA, 21 bp, Artificial Sequence
  Polynucleotide coding gRNA
caatcctctaaaagatgagaa

SEQ ID NO: 138 - DNA, 21 bp, Artificial Sequence
  Polynucleotide coding gRNA
ggctatacaatatggtgattt

SEQ ID NO: 139 - DNA, 21 bp, Artificial Sequence
  Polynucleotide coding gRNA
tttgcagcattagttttctcc

SEQ ID NO: 140 - DNA, 21 bp, Artificial Sequence
  Polynucleotide coding gRNA
aacacaatcaaagtccagatg

SEQ ID NO: 141 - DNA, 21 bp, Artificial Sequence
  Polynucleotide coding gRNA
taaaagcagtaataataagta

SEQ ID NO: 142 - DNA, 21 bp, Artificial Sequence
  Polynucleotide coding gRNA
aagaggtgaatcttatgagtt

SEQ ID NO: 143 - DNA, 21 bp, Artificial Sequence
  Polynucleotide coding gRNA
aaaatcgtggtccatccaaaa

SEQ ID NO: 144 - DNA, 21 bp, Artificial Sequence
  Polynucleotide coding gRNA
gtgtgggcatcaccttgggtc

SEQ ID NO: 145 - DNA, 21 bp, Artificial Sequence
  Polynucleotide coding gRNA
aacagtgtacttgatatcatg

SEQ ID NO: 146 - DNA, 21 bp, Artificial Sequence
  Polynucleotide coding gRNA
gcctagagtgtccaatgtgag

SEQ ID NO: 147 - DNA, 21 bp, Artificial Sequence
  Polynucleotide coding gRNA
tactgtgggataactgacggc

SEQ ID NO: 148 - DNA, 21 bp, Artificial Sequence
  Polynucleotide coding gRNA
caggaagggagctagtgagct

SEQ ID NO: 149 - DNA, 21 bp, Artificial Sequence
  Polynucleotide coding gRNA
agagaagagaaaataggggaa

SEQ ID NO: 150 - DNA, 21 bp, Artificial Sequence
  Polynucleotide coding gRNA
ctccacgccggtagggttaga

SEQ ID NO: 151 - DNA, 21 bp, Artificial Sequence
  Polynucleotide coding gRNA
tgggccgcacgtgtgagtgcc

SEQ ID NO: 152 - DNA, 21 bp, Artificial Sequence
  Polynucleotide coding gRNA
agtttgtagtgtctttccaga

SEQ ID NO: 153 - DNA, 21 bp, Artificial Sequence
  Polynucleotide coding gRNA
ataggttaacaaagatattca

SEQ ID NO: 154 - DNA, 21 bp, Artificial Sequence
  Polynucleotide coding gRNA
gaatgtttaaggtatagttta

SEQ ID NO: 155 - DNA, 21 bp, Artificial Sequence
  Polynucleotide coding gRNA
cagaagagagagagtagtaga

SEQ ID NO: 156 - DNA, 21 bp, Artificial Sequence
  Polynucleotide coding gRNA
tgtttcagcaggggttgaagc

SEQ ID NO: 157 - DNA, 21 bp, Artificial Sequence
  Polynucleotide coding gRNA
ctacaaaataggtgacataac

SEQ ID NO: 158 - DNA, 21 bp, Artificial Sequence
  Polynucleotide coding gRNA
ctataccctagacttattcct

SEQ ID NO: 159 - DNA, 21 bp, Artificial Sequence
  Polynucleotide coding gRNA
tattttccagatgttccaata

SEQ ID NO: 160 - DNA, 21 bp, Artificial Sequence
  Polynucleotide coding gRNA
aggaaacaagcccatgttccc

SEQ ID NO: 161 - DNA, 21 bp, Artificial Sequence
  Polynucleotide coding gRNA
gggaaaatcagacggatattc

SEQ ID NO: 162 - DNA, 21 bp, Artificial Sequence
  Polynucleotide coding gRNA
cctctcctgctgatgatcccc

SEQ ID NO: 163 - DNA, 21 bp, Artificial Sequence
  Polynucleotide coding gRNA
ttaaaatggcgcaaataaatt

SEQ ID NO: 164 - DNA, 21 bp, Artificial Sequence
  Polynucleotide coding gRNA
ttttatgagtctgccaggaat

SEQ ID NO: 165 - DNA, 21 bp, Artificial Sequence
  Polynucleotide coding gRNA
catggcagaaaacagaagaca

SEQ ID NO: 166 - DNA, 21 bp, Artificial Sequence
  Polynucleotide coding gRNA
gaagaaacaattttcactggg

SEQ ID NO: 167 - DNA, 21 bp, Artificial Sequence
  Polynucleotide coding gRNA
tacctatgcctcatgtagaaa

SEQ ID NO: 168 - DNA, 21 bp, Artificial Sequence
  Polynucleotide coding gRNA
gttcagattagctcttaacta

SEQ ID NO: 169 - DNA, 21 bp, Artificial Sequence
  Polynucleotide coding gRNA
aacagtctctgtgatagggca

SEQ ID NO: 170 - DNA, 21 bp, Artificial Sequence
  Polynucleotide coding gRNA
gactatgagactactactgca

SEQ ID NO: 171 - DNA, 21 bp, Artificial Sequence
  Polynucleotide coding gRNA
ccttagcctccttttcacaca

SEQ ID NO: 172 - DNA, 21 bp, Artificial Sequence
  Polynucleotide coding gRNA
gtttctttctacagaatagag

SEQ ID NO: 173 - DNA, 21 bp, Artificial Sequence
  Polynucleotide coding gRNA
atttctgttcttccctcactt

SEQ ID NO: 174 - DNA, 21 bp, Artificial Sequence
  Polynucleotide coding gRNA
taataactgtgtagttataac

SEQ ID NO: 175 - DNA, 21 bp, Artificial Sequence
  Polynucleotide coding gRNA
taaacttcctatttattgtct

SEQ ID NO: 176 - DNA, 21 bp, Artificial Sequence
  Polynucleotide coding gRNA
ataactaatgccagggtgagt

SEQ ID NO: 177 - DNA, 21 bp, Artificial Sequence
  Polynucleotide coding gRNA
atcgtcaggttctgggaccgt

SEQ ID NO: 178 - DNA, 21 bp, Artificial Sequence
  Polynucleotide coding gRNA
tctctttgcaccccaggcatg

SEQ ID NO: 179 - DNA, 21 bp, Artificial Sequence
  Polynucleotide coding gRNA
ttataactaagattctggccc

SEQ ID NO: 180 - DNA, 21 bp, Artificial Sequence
  Polynucleotide coding gRNA
cagatgccagaaaggagactg

SEQ ID NO: 181 - DNA, 21 bp, Artificial Sequence
  Polynucleotide coding gRNA
gaggagaagcggcgataatct

SEQ ID NO: 182 - DNA, 21 bp, Artificial Sequence
  Polynucleotide coding gRNA
gtagaaggctaaatagttacc

SEQ ID NO: 183 - DNA, 21 bp, Artificial Sequence
  Polynucleotide coding gRNA
agtagcacgaacaaaacaagt

SEQ ID NO: 184 - DNA, 21 bp, Artificial Sequence
  Polynucleotide coding gRNA
agataacaataattattactt

SEQ ID NO: 185 - DNA, 21 bp, Artificial Sequence
  Polynucleotide coding gRNA
tcttgactaatctacaccaat

SEQ ID NO: 186 - DNA, 21 bp, Artificial Sequence
  Polynucleotide coding gRNA
gagaaaaatcaggatagaggt

SEQ ID NO: 187 - DNA, 21 bp, Artificial Sequence
  Polynucleotide coding gRNA
ctccacaagcagatgatcaag

SEQ ID NO: 188 - DNA, 21 bp, Artificial Sequence
  Polynucleotide coding gRNA
agatgaggtaaacaggctgga

SEQ ID NO: 189 - DNA, 21 bp, Artificial Sequence
  Polynucleotide coding gRNA
aagttttgtagaaaactaaat

SEQ ID NO: 190 - DNA, 21 bp, Artificial Sequence
  Polynucleotide coding gRNA
atttcatggaaaggttgactt

SEQ ID NO: 191 - DNA, 21 bp, Artificial Sequence
  Polynucleotide coding gRNA
gctttctgctcatacatcccc

SEQ ID NO: 192 - DNA, 21 bp, Artificial Sequence
  Polynucleotide coding gRNA
taccatacaatgatgcttgct

SEQ ID NO: 193 - DNA, 21 bp, Artificial Sequence
  Polynucleotide coding gRNA
aggaaacagacctgtttcctt

SEQ ID NO: 194 - DNA, 21 bp, Artificial Sequence
  Polynucleotide coding gRNA
cacaagatagatagataagat

SEQ ID NO: 195 - DNA, 21 bp, Artificial Sequence
  Polynucleotide coding gRNA
aacagtggggcagttaggatt

SEQ ID NO: 196 - DNA, 21 bp, Artificial Sequence
  Polynucleotide coding gRNA
gactttagctatgcacatgga

SEQ ID NO: 197 - DNA, 21 bp, Artificial Sequence
  Polynucleotide coding gRNA
agaaaaccacagcggctgtgg

SEQ ID NO: 198 - DNA, 21 bp, Artificial Sequence
  Polynucleotide coding gRNA
cgctgaaatttctgagccatg

SEQ ID NO: 199 - DNA, 21 bp, Artificial Sequence
  Polynucleotide coding gRNA
tagtattatctgcaataacaa

SEQ ID NO: 200 - DNA, 21 bp, Artificial Sequence
  Polynucleotide coding gRNA
gaatcaggtgtaatcaattgt

SEQ ID NO: 201 - DNA, 21 bp, Artificial Sequence
  Polynucleotide coding gRNA
tttccaggttttgattgaggt

SEQ ID NO: 202 - DNA, 21 bp, Artificial Sequence
  Polynucleotide coding gRNA
ccctgcaggttggtgtgagca

SEQ ID NO: 203 - DNA, 21 bp, Artificial Sequence
  Polynucleotide coding gRNA
tcacctttggacgtttttaaa

SEQ ID NO: 204 - DNA, 21 bp, Artificial Sequence
  Polynucleotide coding gRNA
ccaaggctcagtaggaaagct

SEQ ID NO: 205 - DNA, 21 bp, Artificial Sequence
  Polynucleotide coding gRNA
aagccgatttagtgcatttgc

SEQ ID NO: 206 - DNA, 21 bp, Artificial Sequence
  Polynucleotide coding gRNA
aattccactctatacacccgg

SEQ ID NO: 207 - DNA, 21 bp, Artificial Sequence
  Polynucleotide coding gRNA
ccagaaagaattcttatagat

SEQ ID NO: 208 - DNA, 21 bp, Artificial Sequence
  Polynucleotide coding gRNA
ctagattttatcattctgtta

SEQ ID NO: 209 - DNA, 21 bp, Artificial Sequence
  Polynucleotide coding gRNA
agtcccctcttgaagaagatg

SEQ ID NO: 210 - DNA, 21 bp, Artificial Sequence
  Polynucleotide coding gRNA
ctatctactggtgataaactg

SEQ ID NO: 211 - DNA, 21 bp, Artificial Sequence
  Polynucleotide coding gRNA
cctggatatcttatgccatgc

SEQ ID NO: 212 - DNA, 21 bp, Artificial Sequence
  Polynucleotide coding gRNA
agactgtagaagcttataaaa

SEQ ID NO: 213 - DNA, 21 bp, Artificial Sequence
  Polynucleotide coding gRNA
aatttagatgtattcattcaa

SEQ ID NO: 214 - DNA, 21 bp, Artificial Sequence
  Polynucleotide coding gRNA
atgtttcttcagttaagacaa

SEQ ID NO: 215 - DNA, 21 bp, Artificial Sequence
  Polynucleotide coding gRNA
atcaaaggtctgttttcagtc

SEQ ID NO: 216 - DNA, 21 bp, Artificial Sequence
  Polynucleotide coding gRNA
gggcaataagctaggggctcc

SEQ ID NO: 217 - DNA, 21 bp, Artificial Sequence
  Polynucleotide coding gRNA
atggtatagccaaactcaaaa

SEQ ID NO: 218 - DNA, 21 bp, Artificial Sequence
  Polynucleotide coding gRNA
tagtaactttagactaagttc

SEQ ID NO: 219 - DNA, 21 bp, Artificial Sequence
  Polynucleotide coding gRNA
tacctccccccactgagaagt

SEQ ID NO: 220 - DNA, 21 bp, Artificial Sequence
  Polynucleotide coding gRNA
ctggcatgaagctctccagcc

SEQ ID NO: 221 - DNA, 21 bp, Artificial Sequence
  Polynucleotide coding gRNA
ctgtaagacctggattatcaa

SEQ ID NO: 222 - DNA, 21 bp, Artificial Sequence
  Polynucleotide coding gRNA
ggtgagcaggtgttggcctga

SEQ ID NO: 223 - DNA, 21 bp, Artificial Sequence
  Polynucleotide coding gRNA
ctggggccctgcttcctacag

SEQ ID NO: 224 - DNA, 21 bp, Artificial Sequence
  Polynucleotide coding gRNA
caaaatgttgtgttagtttaa

SEQ ID NO: 225 - DNA, 21 bp, Artificial Sequence
  Polynucleotide coding gRNA
gccataaaaatttcttctgac

SEQ ID NO: 226 - DNA, 21 bp, Artificial Sequence
  Polynucleotide coding gRNA
gaggctattggatttcatttc

SEQ ID NO: 227 - DNA, 21 bp, Artificial Sequence
  Polynucleotide coding gRNA
gcactcacgaggtcacgaggt

SEQ ID NO: 228 - DNA, 21 bp, Artificial Sequence
  Polynucleotide coding gRNA
ctttcttaaacatagaatcta

SEQ ID NO: 229 - DNA, 21 bp, Artificial Sequence
  Polynucleotide coding gRNA
gaacagtgcaaggataggtgt

SEQ ID NO: 230 - DNA, 21 bp, Artificial Sequence
  Polynucleotide coding gRNA
tggtgccccgggtttacactt

SEQ ID NO: 231 - DNA, 21 bp, Artificial Sequence
  Polynucleotide coding gRNA
cttcatctataggagcctcca

SEQ ID NO: 232 - DNA, 21 bp, Artificial Sequence
  Polynucleotide coding gRNA
ggccttgagtgaggagaaggc

SEQ ID NO: 233 - DNA, 21 bp, Artificial Sequence
  Polynucleotide coding gRNA
ggtgaagtacatattctcata

SEQ ID NO: 234 - DNA, 21 bp, Artificial Sequence
  Polynucleotide coding gRNA
gggctcagttttcccaccagt

SEQ ID NO: 235 - DNA, 21 bp, Artificial Sequence
  Polynucleotide coding gRNA
atacgttttgacggccaatag

SEQ ID NO: 236 - DNA, 21 bp, Artificial Sequence
  Polynucleotide coding gRNA
gtcaaactaaacagccatggg

SEQ ID NO: 237 - DNA, 21 bp, Artificial Sequence
  Polynucleotide coding gRNA
acctatgatgtgatagtttgt

SEQ ID NO: 238 - DNA, 21 bp, Artificial Sequence
  Polynucleotide coding gRNA
taagacctcttaggaagtaga

SEQ ID NO: 239 - DNA, 21 bp, Artificial Sequence
  Polynucleotide coding gRNA
tggaagagtggaaaaaggtgg

SEQ ID NO: 240 - DNA, 21 bp, Artificial Sequence
  Polynucleotide coding gRNA
tttgagaggcaggggcaccag

SEQ ID NO: 241 - DNA, 21 bp, Artificial Sequence
  Polynucleotide coding gRNA
tgtagaatttttaactgttaa

SEQ ID NO: 242 - DNA, 21 bp, Artificial Sequence
  Polynucleotide coding gRNA
gtctaatcttgctctgggtgc

SEQ ID NO: 243 - DNA, 21 bp, Artificial Sequence
  Polynucleotide coding gRNA
cagccaatggtgtaataagct

SEQ ID NO: 244 - DNA, 21 bp, Artificial Sequence
  Polynucleotide coding gRNA
tctgcagaacaggcgcccagt

SEQ ID NO: 245 - DNA, 21 bp, Artificial Sequence
  Polynucleotide coding gRNA
taaagagactcaggagagaag

SEQ ID NO: 246 - DNA, 21 bp, Artificial Sequence
  Polynucleotide coding gRNA
agtctattttgattgttttta

SEQ ID NO: 247 - DNA, 21 bp, Artificial Sequence
  Polynucleotide coding gRNA
gcatcactgaagaatcagcct

SEQ ID NO: 248 - DNA, 21 bp, Artificial Sequence
  Polynucleotide coding gRNA
caagggaggtgcctggttgcc

SEQ ID NO: 249 - DNA, 21 bp, Artificial Sequence
  Polynucleotide coding gRNA
gattttaatcataactgcatg

SEQ ID NO: 250 - DNA, 21 bp, Artificial Sequence
  Polynucleotide coding gRNA
gtcacaagtttctgtttcttg

SEQ ID NO: 251 - DNA, 21 bp, Artificial Sequence
  Polynucleotide coding gRNA
tccatctctgaaatgtggatg

SEQ ID NO: 252 - DNA, 21 bp, Artificial Sequence
  Polynucleotide coding gRNA
taaagggtgcttttcttatta

SEQ ID NO: 253 - DNA, 21 bp, Artificial Sequence
  Polynucleotide coding gRNA
tttgggagtggagagatttgg

SEQ ID NO: 254 - DNA, 21 bp, Artificial Sequence
  Polynucleotide coding gRNA
aggctctcagggaatgagagg